European Patent Application EP 4 681 554 A1, published January 21, 2026. Title: Degradation of harmful biogenic amines in food with a new microbial enzyme derived from Glutamicibacter halophytocola. Applicant: Universität Hohenheim. Application EP. The sequence listing filed with the application follows.

SEQUENCE LISTING (5 sequences)

SEQ ID NO: 1 - protein, 653 aa, Glutamicibacter halophytocola
MEHLHPTTALETAHPLEQITSEEILRTRKILADAGLVEQTTRFAYLGLLDPPKDLLYADAGTEIPRKIRVMLYDPTIPRSLDITICLASAEIESQREIEAATEGQVPVLLEEFDTVEEILANDEGWIKALASRGLSTSQVRVAPLSAGVFDYENEEGKRLLRGLGFVQNSPEDHAWAHPIDRLVAFVDLENRCVDRLIDDGPVPVPDINGNYTDPQVHGELRDDLKAIEITQPDGASFTVDGNHLSWLGWDLRVGFDSREGLVLHQIHHTQDGTRRPLIHRASISEMVVPYGDPSPYRSWQNYFDTGEYLVGRDANSLKLGCDCLGEIHYMSPMVADDFGNPRVIDNGICIHEEDAGIGWKHTDEWAGSNEVRRNRRLVVSFFTTVGNYDYGFYWYLYLDGTIEFEAKATGIVFTAALPHKGYEYASEIAPGLAAPFHQHLFGARLDMMIDGHANAVDELEVVRLPKSEGNPHGNAFTQSRLRLGTEQQAVRDANAAAGRVWQVSNPDSLNHVGEPVGYTLYPQNNPTLAMADDSSIAARAAFTRHDLWVTRFAEGELYAAGDFVNRNPGGAGLPAFVEADRDIDGQDIVLWHSFGLTHFPRPEDWPIMPVDTVGFTLKPHGFFNENPMLNIPASTSSHCSMQAPETEGHCGA

SEQ ID NO: 2 - DNA, 1962 bp, Glutamicibacter halophytocola
  source 1..1962: mol_type = genomic DNA
atggaacaccttcacccaacgacagcgttggagaccgcgcacccactggaacagatcaccagtgaagagatcctgcgtactcgcaagatccttgccgacgccgggctggttgagcagaccacccgtttcgcctacctgggcttgctggatccacccaaggacctgctctatgccgatgctggcacagagattccgcgcaagattcgtgtgatgctctacgatccgaccatcccccgctccctggacatcacgatctgcctggccagcgccgagatagaatcacagcgcgaaatcgaagcagcgacagagggacaagttccggtgctgcttgaagaattcgacaccgtcgaagaaatcctggccaacgacgaaggatggatcaaggccttggccagccgcggactgagcacatcccaggttcgagtcgcaccgctgtcagcaggtgtcttcgactacgagaacgaagaaggaaaacgcctattgcgcggactgggcttcgtgcagaattcccctgaggaccacgcttgggcccaccccatcgatcgcttggtggcctttgtcgacctcgaaaaccgttgcgttgaccggctcatcgatgatggccctgttccagttcccgacatcaacggaaactacactgatccacaagttcatggtgagctgcgcgatgatctcaaggccatcgaaatcacccagccagatggagccagcttcaccgtggatggcaaccacctctcgtggctcggctgggatctgcgcgtcggctttgactcacgcgaaggactcgtactccaccagatccaccacacgcaagacggcacgcgtcgcccgctgatccaccgcgcatccatctccgaaatggtagtgccctacggcgatccgtccccttaccggagctggcagaactatttcgacaccggagaatatttggtgggacgcgacgcgaactcactgaagctcggctgcgactgcctcggagaaatccactacatgtctcccatggttgccgacgattttggcaatcctcgcgtcatcgacaacggcatctgcattcacgaggaagacgccggaatcggatggaagcacaccgatgagtgggccggatccaacgaagtgcgccgcaaccggcgcctggtggtttccttcttcaccaccgtgggcaattatgactacggtttctactggtacctgtacctcgacggcaccatcgagtttgaagccaaggccacgggcatcgtcttcaccgcggcgttgccgcacaagggttacgagtacgcctcagaaatcgcgccgggcttggctgcgccattccaccagcatctctttggcgcacgccttgacatgatgatcgacgggcacgccaacgctgttgacgagctagaagtagtccggttaccgaagtccgaaggcaatccacacggcaacgccttcacccaaagccggctgcgtttgggcaccgagcagcaggcggtacgcgacgccaatgcagcggcgggacgcgtatggcaggtgagcaaccccgattccctgaatcacgtgggcgagccggtgggctacacgttgtacccgcagaacaatccgacgctggctatggctgacgactcgtccatcgctgcccgtgccgcctttacccgacacgacctctgggtcacgcgctttgccgaaggcgagctctatgcagccggcgacttcgtcaaccgcaatccaggcggggcggggcttcctgccttcgtcgaggccgaccgggatatcgacggacaagatatcgtgttgtggcactcctttggcctgacccacttccctcgccccgaggactggcccatcatgccagtggataccgtagggttcacgctgaagccacacggtttcttcaatgaaaacccgatgctcaatatccctgcctcgacaagctcgcactgttccatgcaagctcctgaaaccgaaggacactgcggagcctag

SEQ ID NO: 3 - DNA, 1962 bp, synthetic construct
  source 1..1962: mol_type = other DNA
atggaacacttgcacccaactactgctttggaaactgctcaccctttggagcagattacctccgaagagatcctgagaaccagaaagattttggctgacgccggtttggttgagcagactactagatttgcctacttgggtttgctggacccaccaaaggatttgttgtacgctgatgctggtactgagatcccaagaaagatcagagtcatgctgtacgacccaactatcccaagatccttggacattaccatctgtttggcttccgctgagattgagtcccagagagaaattgaagctgctaccgaaggtcaggtcccagttttgttggaagagttcgacaccgtggaagagatcttggctaacgacgaaggttggatcaaggctttggcttctagaggtttgtccacctctcaggttagagttgctccattgtctgctggtgttttcgactacgaaaacgaggaaggtaagagactgttgagaggtttgggtttcgttcagaactctccagaagatcacgcttgggctcacccaattgatagattggttgccttcgtcgacttggagaacagatgtgtcgacagattgattgacgacggtccagttccagttcctgacatcaacggtaactacactgacccacaagttcacggtgagttgagagatgacttgaaggctatcgagatcactcaaccagacggtgcttctttcactgttgacggtaaccacttgtcttggcttggttgggatttgagagttggtttcgactccagagaaggtttggtcttgcaccagattcaccacactcaagacggtactagaaggccattgattcacagagcttccatttccgagatggtcgttccatacggtgatccatctccatacagatcctggcagaactacttcgacactggtgagtacttggttggtagagatgccaactccttgaagttgggttgtgactgtttgggtgagatccactacatgtccccaatggttgctgatgacttcggtaacccaagagtcatcgacaacggtatctgtatccacgaagaggacgctggtattggttggaagcacactgatgaatgggctggttctaacgaggtcagaagaaacagaagattggtcgtttccttcttcaccaccgttggtaactacgactacggtttctactggtacttgtacctggacggaactatcgagttcgaggctaaggctactggtatcgttttcactgctgctttgccacacaagggttacgaatacgcttctgagattgctccaggtttggctgctccatttcaccaacatttgttcggtgccagactggacatgatgattgatggtcatgctaacgccgttgacgagttggaggttgttagattgccaaagtctgagggtaacccacacggtaacgctttcactcagtccagattgagattgggtactgagcagcaggctgtcagagatgctaatgctgctgctggtagagtttggcaggtttctaacccagactctttgaaccacgttggtgagccagttggttacactctgtacccacaaaacaaccctactttggctatggctgacgactcttccattgctgctagagctgctttcactagacacgatttgtgggtgactagattcgctgagggtgagttgtatgctgccggtgatttcgttaacagaaacccaggtggtgctggtttgccagcttttgttgaagctgacagagacattgacggtcaggacatcgttttgtggcattcctttggtctgactcacttcccaagacctgaggactggccaattatgccagttgacactgttggtttcaccttgaagccacacggtttcttcaacgagaacccaatgttgaatatcccagcctccacttcttcccactgttctatgcaagctccagaaactgaaggtcactgtggtgcttaa

SEQ ID NO: 4 - DNA, 22 bp, synthetic construct
  source 1..22: mol_type = other DNA
atggaacaccttcacccaacga

SEQ ID NO: 5 - DNA, 30 bp, synthetic construct
  source 1..30: mol_type = other DNA
ctaggctccgcagtgtccttcggtttcagg